European Patent Application EP 4 636 402 A1, published October 22, 2025. Title: Highly Sensitive Detection Method for Cancer cell-Derived Extracellular Vesicles Using Fusion Reaction with Liposomes. Applicant: INSTITUTE FOR BASIC SCIENCE. The sequence listing filed with the application follows.

SEQUENCE LISTING (3 sequences)

SEQ ID NO: 1 - DNA, 36 bp, synthetic construct
  source 1..36: mol_type = other DNA
agctgcatgatgagctgcacggtggcagctcatcat

SEQ ID NO: 2 - DNA, 35 bp, synthetic construct
  source 1..35: mol_type = other DNA
ttggcccgcccaaaatctgtgattagatttgggcg

SEQ ID NO: 3 - DNA, 37 bp, synthetic construct
  source 1..37: mol_type = other DNA
tcaacatcagtctgataagctagtattatcagactga